European Patent Specification EP 3 967 757 B1, published January 31, 2024. Title: ALPHA-AMYLASE VARIANTS. Applicant: DANISCO US INC. Application EP Divisional of EP13729864.2. The sequence listing filed with the application follows.

SEQUENCE LISTING (4 sequences)

SEQ ID NO: 1 - protein, 485 aa, Cytophaga sp.
  misc_feature: amino acid sequence of the mature form of Cytophaga sp. amylase (CspAmy2)
AATNGTMMQYFEWYVPNDGQQWNRLRTDAPYLSSVGITAVWTPPAYKGTSQADVGYGPYDLYDLGEFNQKGTVRTKYGTKGELKSAVNTLHSNGIQVYGDVVMNHKAGADYTENVTAVEVNPSNRNQETSGEYNIQAWTGFNFPGRGTTYSNFKWQWFHFDGTDWDQSRSLSRIFKFRGTGKAWDWEVSSENGNYDYLMYADIDYDHPDVVNEMKKWGVWYANEVGLDGYRLDAVKHIKFSFLKDWVDNARAATGKEMFTVGEYWQNDLGALNNYLAKVNYNQSLFDAPLHYNFYAASTGGGYYDMRNILNNTLVASNPTKAVTLVENHDTQPGQSLESTVQPWFKPLAYAFILTRSGGYPSVFYGDMYGTKGTTTREIPALKSKIEPLLKARKDYAYGTQRDYIDNPDVIGWTREGDSTKAKSGLATVITDGPGGSKRMYVGTSNAGEIWYDLTGNRTDKITIGSDGYATFPVNGGSVSVWVQQ

SEQ ID NO: 2 - protein, 483 aa, Artificial Sequence
  Synthetic amino acid: sequence of the mature CspAmy2-v1 amylase polypeptide
AATNGTMMQYFEWYVPNDGQQWNRLRTDAPYLSSVGITAVWTPPAYKGTSQADVGYGPYDLYDLGEFNQKGTVRTKYGTKGELKSAVNTLHSNGIQVYGDVVMNHKAGADYTENVTAVEVNPSNRNQETSGEYNIQAWTGFNFPGRGTTYSNFKWQWFHFDGTDWDQSRSLSRIFKFTGKAWDWEVSSENGNYDYLMYADIDYDHPDVVNEMKKWGVWYANEVGLDGYRLDAVKHIKFSFLKDWVDNARAATGKEMFTVGEYWQNDLGALNNYLAKVNYNQSLFDAPLHYNFYAASTGGGYYDMRNILNNTLVASNPTKAVTLVENHDTQPGQSLESTVQPWFKPLAYAFILTRSGGYPSVFYGDMYGTKGTTTREIPALKSKIEPLLKARKDYAYGTQRDYIDNPDVIGWTREGDSTKAKSGLATVITDGPGGSKRMYVGTSNAGEIWYDLTGNRTDKITIGSDGYATFPVNGGSVSVWVQQ

SEQ ID NO: 3 - protein, 512 aa, Artificial Sequence
  Synthetic amino acid: precursor form of the CspAmy2-v1 polypeptide produced from the pHPLT02-CspAmy2-v1 vector
MKQQKRLYARLLTLLFALIFLLPHSAASAAATNGTMMQYFEWYVPNDGQQWNRLRTDAPYLSSVGITAVWTPPAYKGTSQADVGYGPYDLYDLGEFNQKGTVRTKYGTKGELKSAVNTLHSNGIQVYGDVVMNHKAGADYTENVTAVEVNPSNRNQETSGEYNIQAWTGFNFPGRGTTYSNFKWQWFHFDGTDWDQSRSLSRIFKFTGKAWDWEVSSENGNYDYLMYADIDYDHPDVVNEMKKWGVWYANEVGLDGYRLDAVKHIKFSFLKDWVDNARAATGKEMFTVGEYWQNDLGALNNYLAKVNYNQSLFDAPLHYNFYAASTGGGYYDMRNILNNTLVASNPTKAVTLVENHDTQPGQSLESTVQPWFKPLAYAFILTRSGGYPSVFYGDMYGTKGTTTREIPALKSKIEPLLKARKDYAYGTQRDYIDNPDVIGWTREGDSTKAKSGLATVITDGPGGSKRMYVGTSNAGEIWYDLTGNRTDKITIGSDGYATFPVNGGSVSVWVQQ

SEQ ID NO: 4 - DNA, 1536 bp, Artificial Sequence
  synthetic DNA fragment, CspAmy2-v1 DNA, encoding CspAmy2-v1
atgaaacaacaaaaacggctttacgcccgattgctgacgctgttatttgcgctcatcttcttgctgcctcattctgcagctagcgcagcagcgacaaacggaacaatgatgcagtatttcgagtggtatgtacctaacgacggccagcaatggaacagactgagaacagatgccccttacttgtcatctgttggtattacagcagtatggacaccgccggcttataagggcacgtctcaagcagatgtggggtacggcccgtacgatctgtatgatttaggcgagtttaatcaaaaaggtacagtcagaacgaagtatggcacaaaaggagaacttaaatctgctgttaacacgctgcattcaaatggaatccaagtgtatggtgatgtcgtgatgaatcataaagcaggtgctgattatacagaaaacgtaacggcggtggaggtgaatccgtctaatagaaatcaggaaacgagcggcgaatataatattcaggcatggacaggcttcaactttccgggcagaggaacaacgtattctaacttcaaatggcagtggttccattttgatggaacggattgggaccagagcagaagcctctctagaatcttcaaattcacgggaaaggcgtgggactgggaggtttcttcagaaaacggaaattatgactatctgatgtacgcggacattgattatgaccatccggatgtcgtgaatgaaatgaaaaagtggggcgtctggtatgccaacgaagttgggttagatggatacagacttgacgcggtcaaacatattaaatttagctttctcaaagactgggtggataacgcaagagcagcgacgggaaaagaaatgtttacggttggcgaatattggcaaaatgatttaggggccctgaataactacctggcaaaggtaaattacaaccaatctctttttgatgcgccgttgcattacaacttttacgctgcctcaacagggggtggatattacgatatgagaaatattcttaataacacgttagtcgcaagcaatccgacaaaggctgttacgttagttgagaatcatgacacacagcctggacaatcactggaatcaacagtccaaccgtggtttaaaccgttagcctacgcgtttattctcacgagaagcggaggctatccttctgtattttatggagatatgtacggtacaaaaggaacgacaacaagagagatccctgctcttaaatctaaaatcgaacctttgcttaaggctagaaaagactatgcttatggaacacagagagactatattgataacccggatgtcattggctggacgagagaaggggactcaacgaaagccaagagcggtctggccacagtgattacagatgggccgggcggttcaaaaagaatgtatgttggcacgagcaatgcgggtgaaatctggtatgatttgacagggaatagaacagataaaatcacgattggaagcgatggctatgcaacatttcctgtcaatgggggctcagtttcagtatgggtgcagcaa